European Patent Application EP 4 570 262 A1, published June 18, 2025. Title: CHIMERIC ANTIGEN RECEPTOR DIRECTED AGAINST THE CHEMOKINE RECEPTOR CCR7. Applicant: Max Delbrück Center. The sequence listing filed with the application follows.

SEQUENCE LISTING (46 sequences)

SEQ ID NO: 1 - protein, 8 aa, Rattus norvegicus
GFTFSNAA

SEQ ID NO: 2 - protein, 10 aa, Rattus norvegicus
IRTKPNNFAT

SEQ ID NO: 3 - protein, 9 aa, Rattus norvegicus
TAGKDYFAY

SEQ ID NO: 4 - protein, 11 aa, Rattus norvegicus
KSLLFSDGKTY

SEQ ID NO: 5 - skipped

SEQ ID NO: 6 - protein, 9 aa, Rattus norvegicus
QQFLEFPFT

SEQ ID NO: 7 - protein, 118 aa, synthetic construct
XVQLVESGGGLVQPXXSLKXSCAASGFTFSXXAMXWVRQAXGKGLEWVXRIRXKXNXXATXYAXSVKGRFTISRDDSKXXXYLQMXXLKTEDTAXYYCTAGKDYFAYWGQGTLVTVSS

SEQ ID NO: 8 - protein, 113 aa, synthetic construct
DIVMTQXXLXXPVXXGEXASIXCXSSXSLLXSDGXTYLXWYLQXPGQSPQXLIYXXSXRASGVXDRFSGSGSGTDFTLKISRVEAEDVGVYYCXQXXEFPFTFGSGTKLEIKR

SEQ ID NO: 9 - protein, 118 aa, synthetic construct
EVQLVESGGGLVQPGGSLKLSCAASGFTFSNAAMHWVRQASGKGLEWVGRIRTKPNNFATAYAASVKGRFTISRDDSKNTAYLQMNKLKTEDTAVYYCTAGKDYFAYWGQGTLVTVSS

SEQ ID NO: 10 - protein, 118 aa, synthetic construct
EVQLVESGGGLVQPKESLKLSCAASGFTFSNAAMYWVRQAPGKGLEWVARIRTKPNNFATYYADSVKGRFTISRDDSKSMAYLQMNKLKTEDTAMYYCTAGKDYFAYWGQGTLVTVSS

SEQ ID NO: 11 - protein, 118 aa, synthetic construct
EVQLVESGGGLVQPGGSLKLSCAASGFTFSNAAMYWVRQAPGKGLEWVARIRTKPNNFATYYADSVKGRFTISRDDSKSMAYLQMNKLKTEDTAMYYCTAGKDYFAYWGQGTLVTVSS

SEQ ID NO: 12 - protein, 118 aa, synthetic construct
EVQLVESGGGLVQPKESLKLSCAASGFTFSNAAMHWVRQASGKGLEWVGRIRTKPNNFATYYADSVKGRFTISRDDSKSMAYLQMNKLKTEDTAMYYCTAGKDYFAYWGQGTLVTVSS

SEQ ID NO: 13 - protein, 118 aa, synthetic construct
EVQLVESGGGLVQPKESLKLSCAASGFTFSNAAMYWVRQAPGKGLEWVARIRTKPNNFATAYAASVKGRFTISRDDSKSMAYLQMNKLKTEDTAMYYCTAGKDYFAYWGQGTLVTVSS

SEQ ID NO: 14 - protein, 118 aa, synthetic construct
EVQLVESGGGLVQPKESLKLSCAASGFTFSNAAMYWVRQAPGKGLEWVARIRTKPNNFATYYADSVKGRFTISRDDSKNTAYLQMNKLKTEDTAVYYCTAGKDYFAYWGQGTLVTVSS

SEQ ID NO: 15 - protein, 118 aa, Homo sapiens
EVQLVESGGGLVQPGGSLKLSCAASGFTFSGSAMHWVRQASGKGLEWVGRIRSKANSYATAYAASVKGRFTISRDDSKNTAYLQMNSLKTEDTAVYYCTAGKDYFAYWGQGTLVTVSS

SEQ ID NO: 16 - protein, 117 aa, Rattus norvegicus
VQLVESGGGLVQPKESLKISCAASGFTFSNAAMYWVRQAPGKGLEWVARIRTKPNNFATYYADSVKGRFTISRDDSKSMVYLQMDKLKTEDTAMYYCTAGKDYFAYWGQGTLVTVSS

SEQ ID NO: 17 - protein, 113 aa, synthetic construct
DIVMTQTPLSLPVTPGEPASISCRSSKSLLFSDGKTYLDWYLQKPGQSPQLLIYWMSYRASGVPDRFSGSGSGTDFTLKISRVEAEDVGVYYCQQFLEFPFTFGSGTKLEIKR

SEQ ID NO: 18 - protein, 113 aa, synthetic construct
DIVMTQTPLSLPVTPGEPASISCRSSKSLLFSDGKTYLNWYLQKPGQSPQLLIYWMSYRASGVPDRFSGSGSGTDFTLKISRVEAEDVGVYYCQQFLEFPFTFGSGTKLEIKR

SEQ ID NO: 19 - protein, 113 aa, synthetic construct
DIVMTQGALPNPVTSGESASISCQSSKSLLFSDGKTYLDWYLQKPGQSPQFLIYWMSTRASGVSDRFSGSGSGTDFTLKISRVEAEDVGVYYCQQFLEFPFTFGSGTKLEIKR

SEQ ID NO: 20 - protein, 113 aa, synthetic construct
DIVMTQGALPNPVTSGESASISCQSSKSLLFSDGKTYLNWYLQKPGQSPQFLIYWMSTRASGVSDRFSGSGSGTDFTLKISRVEAEDVGVYYCQQFLEFPFTFGSGTKLEIKR

SEQ ID NO: 21 - protein, 113 aa, synthetic construct
DIVMTQTPLSNPVTSGESASISCQSSKSLLFSDGKTYLNWYLQKPGQSPQFLIYWMSTRASGVSDRFSGSGSGTDFTLKISRVEAEDVGVYYCQQFLEFPFTFGSGTKLEIKR

SEQ ID NO: 22 - protein, 113 aa, synthetic construct
DIVMTQGALPLPVTPGESASISCQSSKSLLFSDGKTYLNWYLQKPGQSPQFLIYWMSTRASGVSDRFSGSGSGTDFTLKISRVEAEDVGVYYCQQFLEFPFTFGSGTKLEIKR

SEQ ID NO: 23 - protein, 113 aa, synthetic construct
DIVMTQGALPNPVTSGEPASISCRSSKSLLFSDGKTYLNWYLQKPGQSPQFLIYWMSTRASGVSDRFSGSGSGTDFTLKISRVEAEDVGVYYCQQFLEFPFTFGSGTKLEIKR

SEQ ID NO: 24 - protein, 113 aa, synthetic construct
DIVMTQGALPNPVTSGESASISCQSSKSLLFSDGKTYLNWYLQKPGQSPQLLIYWMSYRASGVPDRFSGSGSGTDFTLKISRVEAEDVGVYYCQQFLEFPFTFGSGTKLEIKR

SEQ ID NO: 25 - protein, 113 aa, synthetic construct; identical to SEQ ID NO: 18

SEQ ID NO: 26 - protein, 114 aa, Homo sapiens
DIVMTQTPLSLPVTPGEPASISCRSSQSLLDSDDGNTYLDWYLQKPGQSPQLLIYTLSYRASGVPDRFSGSGSGTDFTLKISRVEAEDVGVYYCMQRIEFPFTFGSGTKLEIKR

SEQ ID NO: 27 - protein, 112 aa, Rattus norvegicus
DIVMTQGALPNPVPSGESASITCQSSKSLLFSDGKTYLNWYLQRPGQSPQFLIYWMSTRASGVSDRFSGSGSGTDFTLKISRVEAEDVGVYYCQQFLEFPFTFGSGTKLEIK

SEQ ID NO: 28 - protein, 18 aa, synthetic construct
GSTSGSGKPGSGEGSTKG

SEQ ID NO: 29 - protein, 237 aa, synthetic construct
PAEPKSPDKTHTCPPCPAPPVAGPSVFLFPPKPKDTLMIARTPEVTCVVVDVSHEDPEVKFNWYVDGVEVHNAKTKPREEQYNSTYRVVSVLTVLHQDWLNGKEYKCKVSNKALPAPIEKTISKAKGQPREPQVYTLPPSRDELTKNQVSLTCLVKGFYPSDIAVEWESNGQPENNYKTTPPVLDSDGSFFLYSKLTVDKSRWQQGNVFSCSVMHEALHNHYTQKSLSLSPGKKDPK

SEQ ID NO: 30 - protein, 27 aa, synthetic construct
FWVLVVVGGVLACYSLLVTVAFIIFWV

SEQ ID NO: 31 - protein, 42 aa, synthetic construct
RSKRSRLLHSDYMNMTPRRPGPTRKHYQPYAPPRDFAAYRSL

SEQ ID NO: 32 - protein, 113 aa, synthetic construct
LRVKFSRSADAPAYQQGQNQLYNELNLGRREEYDVLDKRRGRDPEMGGKPRRKNPQEGLYNELQKDKMAEAYSEIGMKGERRRGKGHDGLYQGLSTATKDTYDALHMQALPPR

SEQ ID NO: 33 - protein, 21 aa, synthetic construct
MDFQVQIFSFLLISASVIMSR

SEQ ID NO: 34 - protein, 688 aa, Rattus norvegicus
MDFQVQIFSFLLISASVIMSRAVQLVESGGGLVQPKESLKISCAASGFTFSNAAMYWVRQAPGKGLEWVARIRTKPNNFATYYADSVKGRFTISRDDSKSMVYLQMDKLKTEDTAMYYCTAGKDYFAYWGQGTLVTVSSGSTSGSGKPGSGEGSTKGDIVMTQGALPNPVPSGESASITCQSSKSLLFSDGKTYLNWYLQRPGQSPQFLIYWMSTRASGVSDRFSGSGSGTDFTLKISRVEAEDVGVYYCQQFLEFPFTFGSGTKLEIKRPAEPKSPDKTHTCPPCPAPPVAGPSVFLFPPKPKDTLMIARTPEVTCVVVDVSHEDPEVKFNWYVDGVEVHNAKTKPREEQYNSTYRVVSVLTVLHQDWLNGKEYKCKVSNKALPAPIEKTISKAKGQPREPQVYTLPPSRDELTKNQVSLTCLVKGFYPSDIAVEWESNGQPENNYKTTPPVLDSDGSFFLYSKLTVDKSRWQQGNVFSCSVMHEALHNHYTQKSLSLSPGKKDPKFWVLVVVGGVLACYSLLVTVAFIIFWVRSKRSRLLHSDYMNMTPRRPGPTRKHYQPYAPPRDFAAYRSLRVKFSRSADAPAYQQGQNQLYNELNLGRREEYDVLDKRRGRDPEMGGKPRRKNPQEGLYNELQKDKMAEAYSEIGMKGERRRGKGHDGLYQGLSTATKDTYDALHMQALPPR

SEQ ID NO: 35 - protein, 17 aa, synthetic construct
SSGGGGSGGGGSGGGGS

SEQ ID NO: 36 - protein, 235 aa, synthetic construct
PAEPKSPDKTHTCPPCPAPPVAGPSVFLFPPKPKDTLMIARTPEVTCVVVDVSHEDPEVKFNWYVDGVEVHNAKTKPREEQYNSTYRVVSVLTVLHQDWLNGKEYKCKVSNKALPAPIEKTISKAKGQPREPQVYTLPPSRDELTKNQVSLTCLVKGFYPSDIAVEWESNGQPENNYKTTPPVLDSDGSFFLYSKLTVDKSRWQQGNVFSCSVMHEALHNHYTQKSLSSLSPGKK

SEQ ID NO: 37 - protein, 229 aa, synthetic construct
ESKYGPPCPPCPAPEFEGGPSVFLFPPKPKDTLMISRTPEVTCVVVDVSQEDPEVQFNWYVDGVEVHNAKTKPREEQFNSTYRVVSVLTVLHQDWLNGKEYKCKVSNKGLPSSIEKTISKAKGQPREPQVYTLPPSQEEMTKNQVSLTCLVKGFYPSDIAVEWESNGQPENNYKTTPPVLDSDGSFFLYSRLTVDKSRWQEGNVFSCSVMHEALHNHYTQKSLSLSLGK

SEQ ID NO: 38 - protein, 118 aa, synthetic construct
ESKYGPPCPPCPGQPREPQVYTLPPSQEEMTKNQVSLTCLVKGFYPSDIAVEWESNGQPENNYKTTPPVLDSDGSFFLYSRLTVDKSRWQEGNVFSCSVMHEALHNHYTQKSLSLSLG

SEQ ID NO: 39 - protein, 12 aa, synthetic construct
ESKYGPPCPPCP

SEQ ID NO: 40 - protein, 24 aa, synthetic construct
IYIWAPLAGTCGVLLLSLVITLYC

SEQ ID NO: 41 - protein, 42 aa, synthetic construct
KRGRKKLLYIFKQPFMRPVQTTQEEDGCSCRFPEEEEGGCEL

SEQ ID NO: 42 - DNA, 2067 bp, Rattus norvegicus
  source 1..2067: mol_type = genomic DNA
atggattttcaggtgcagatcttcagcttcctgctgatctccgccagcgtgatcatgagcagagccgtgcagctggtggaatctggcggaggactggtgcagcctaaagagagcctgaagatcagctgtgccgccagcggcttcacctttagcaatgccgccatgtactgggtccgacaggcccctggaaaaggcctggaatgggttgcccggatcaggaccaagcctaacaacttcgccacctactacgccgacagcgtgaagggcagattcaccatcagccgggacgacagcaagagcatggtgtacctgcagatggacaagctgaaaaccgaggacaccgctatgtactactgcaccgccggcaaggactacttcgcctattggggacagggcaccctggtcacagtgtctagcggctctacaagcggctctggcaaacctggatctggcgagggaagcaccaagggcgatatcgtgatgacacagggcgctctgcccaatcctgtgccttctggcgagagcgcctctatcacctgtcagagcagcaagtccctgctgttcagcgacggcaagacctacctgaactggtatctgcagaggcccggacagagccctcagttcctgatctactggatgagcaccagagccagcggcgtgtccgatagattttctggcagcggctccggcaccgacttcaccctgaagattagcagagtggaagccgaggacgtgggcgtgtactattgccagcagttcctggaattcccattcaccttcggcagcggcaccaagctggaaatcaagagacccgccgagcccaagagccccgacaagacccatacctgccctccatgtcctgcccctccagtggctggccctagcgtgttcctgttccccccaaagcccaaggacaccctgatgatcgcccggacccctgaagtgacctgcgtggtggtggatgtgtcccacgaggatcccgaagtgaagttcaattggtacgtggacggcgtggaagtgcacaacgccaagaccaagcccagagaggaacagtacaacagcacctaccgggtggtgtctgtgctgaccgtgctgcatcaggactggctgaacggcaaagagtacaagtgcaaggtgtccaacaaggccctgcctgcccccatcgagaaaaccatctccaaggccaagggacagccccgcgagccccaggtgtacacactgcctccaagcagggacgagctgaccaagaaccaggtcagcctgacctgcctggtcaaaggcttctatcccagcgacatcgccgtggagtgggagagcaatgggcagccggagaacaactacaagaccacgcctcccgtgctggactccgacggctccttcttcctctacagcaagctcaccgtggacaagagcaggtggcagcaggggaacgtcttctcatgctccgtgatgcatgaggctctgcacaaccactacacgcagaagagcctctccctgtctccgggtaaaaaagatcccaaattttgggtgctggtggtggttggtggagtcctggcttgctatagcttgctagtaacagtggcctttattattttctgggtgaggagtaagaggagcaggctcctgcacagtgactacatgaacatgactccccgccgccccgggcccacccgcaagcattaccagccctatgccccaccacgcgacttcgcagcctatcgctccctgagagtgaagttcagcaggagcgcagacgcccccgcgtaccagcagggccagaaccagctctataacgagctcaatctaggacgaagagaggagtacgatgttttggacaagagacgtggccgggaccctgagatggggggaaagccgagaaggaagaaccctcaggaaggcctgtacaatgaactgcagaaagataagatggcggaggcctacagtgagattgggatgaaaggcgagcgccggaggggcaaggggcacgatggcctttaccagggtctcagtacagccaccaaggacacctacgacgcccttcacatgcaggccctgccccctcgctga

SEQ ID NO: 43 - DNA, 355 bp, Rattus norvegicus
  source 1..355: mol_type = genomic DNA
gccgtgcagcttgttgagtctggtggaggattggtgcagcctaaggagtcattgaaaatctcatgtgcagcctctggattcaccttcagtaatgctgccatgtactgggtccgccaggctccaggaaagggtctggaatgggttgctcgcataagaactaaacctaataattttgcaacatattatgctgactcagtgaaaggcagattcaccatctccagagatgattcaaaaagcatggtctacctacaaatggataagttgaaaactgaggacacagccatgtattattgtacagctgggaaggattactttgcttactggggccaaggcactctggtcactgtctcttcag

SEQ ID NO: 44 - DNA, 351 bp, synthetic construct
  source 1..351: mol_type = other DNA
gccgtgcagctggtggaatctggcggaggactggtgcagcctaaagagagcctgaagatcagctgtgccgccagcggcttcacctttagcaatgccgccatgtactgggtccgacaggcccctggaaaaggcctggaatgggttgcccggatcaggaccaagcctaacaacttcgccacctactacgccgacagcgtgaagggcagattcaccatcagccgggacgacagcaagagcatggtgtacctgcagatggacaagctgaaaaccgaggacaccgctatgtactactgcaccgccggcaaggactacttcgcctattggggacagggcaccctggtcacagtgtct

SEQ ID NO: 45 - DNA, 337 bp, Rattus norvegicus
  source 1..337: mol_type = genomic DNA
gatattgtgatgacccagggtgcactccccaatcctgtcccttctggagagtcagcttccatcacctgccagtctagcaagagtctgctgttcagcgatggcaagacatacttgaattggtatctgcagaggccaggacagtctcctcagttcctgatctattggatgtctacccgtgcatcaggagtctcagacaggttcagtggcagtgggtcaggaacagatttcacactgaaaatcagtagagtggaggctgaggatgtgggtgtgtattactgtcagcaatttctagagtttccattcacgttcggctcagggacgaagttggaaataaaac

SEQ ID NO: 46 - DNA, 335 bp, synthetic construct
  source 1..335: mol_type = other DNA
gatatcgtgatgacacagggcgctctgcccaatcctgtgccttctggcgagagcgcctctatcacctgtcagagcagcaagtccctgctgttcagcgacggcaagacctacctgaactggtatctgcagaggcccggacagagccctcagttcctgatctactggatgagcaccagagccagcggcgtgtccgatagattttctggcagcggctccggcaccgacttcaccctgaagattagcagagtggaagccgaggacgtgggcgtgtactattgccagcagttcctggagttcccattcaccttcggcagcggcaccaagctggaaatcaa